European Patent Specification EP 3 828 197 B1, published October 2, 2024. Title: MURINE ANTI-NY-ESO-1 T CELL RECEPTORS. Applicant: THE UNITED STATES OF AMERICA, AS REPRESENTED BY THE SECRETARY, DEPARTMENT OF HEALTH AND HUMAN SERVICES. Application not yet assigned. The sequence listing filed with the application follows.

SEQUENCE LISTING (28 sequences)

SEQ ID NO: 1 - protein, 180 aa, Homo sapiens
MQAEGRGTGGSTGDADGPGGPGIPDGPGGNAGGPGEAGATGGRGPRGAGAARASGPGGGAPRGPHGGAASGLNGCCRCGARGPESRLLEFYLAMPFATPMEAELARRSLAQDAPPLPVPGVLLKEFTVSGNILTIRLTAADHRQLQLSISSCLQQLSLLMWITQCFLPVFLAQPPSGQRR

SEQ ID NO: 2 - protein, 9 aa, Homo sapiens
SLLMWITQC

SEQ ID NO: 3 - protein, 8 aa, Mus musculus
ATSIGYPN

SEQ ID NO: 4 - protein, 7 aa, Mus musculus
VITAGQK

SEQ ID NO: 5 - protein, 12 aa, Mus musculus
CALWSGSWQLIF

SEQ ID NO: 6 - protein, 5 aa, Mus musculus
KGHPV

SEQ ID NO: 7 - protein, 6 aa, Mus musculus
FQNQEV

SEQ ID NO: 8 - protein, 11 aa, Mus musculus
CASRDSPEQYF

SEQ ID NO: 9 - protein, 136 aa, Mus musculus
MTLKMDSSPGFVAVILLILGRTHGDSVTQTEGQVTVSESKSLIINCTYSATSIGYPNLFWYVRYPGEGLQLLLKVITAGQKGSSRGFEATYNKEATSFHLQKASVQESDSAVYYCALWSGSWQLIFGSGTQLTVMP

SEQ ID NO: 10 - protein, 131 aa, Mus musculus
MATRLLCYTVLCLLGARILNSKVIQTPRYLVKGQGQKAKMRCIPEKGHPVVFWYQQNKNNEFKFLINFQNQEVLQQIDMTEKRFSAECPSNSPCSLEIQSSEAGDSALYLCASRDSPEQYFGPGTRLTVLE

SEQ ID NO: 11 - protein, 273 aa, Mus musculus
MTLKMDSSPGFVAVILLILGRTHGDSVTQTEGQVTVSESKSLIINCTYSATSIGYPNLFWYVRYPGEGLQLLLKVITAGQKGSSRGFEATYNKEATSFHLQKASVQESDSAVYYCALWSGSWQLIFGSGTQLTVMPDIQNPEPAVYQLKDPRSQDSTLCLFTDFDSQINVPKTMESGTFITDKTVLDMKAMDSKSNGAIAWSNQTSFTCQDIFKETNATYPSSDVPCDATLTEKSFETDMNLNFQNLSVMGLRILLLKVAGFNLLMTLRLWSS

SEQ ID NO: 12 - protein, 303 aa, Mus musculus
MATRLLCYTVLCLLGARILNSKVIQTPRYLVKGQGQKAKMRCIPEKGHPVVFWYQQNKNNEFKFLINFQNQEVLQQIDMTEKRFSAECPSNSPCSLEIQSSEAGDSALYLCASRDSPEQYFGPGTRLTVLEDLRNVTPPKVSLFEPSKAEIANKQKATLVCLARGFFPDHVELSWWVNGKEVHSGVSTDPQAYKESNYSYCLSSRLRVSATFWHNPRNHFRCQVQFHGLSEEDKWPEGSPKPVTQNISAEAWGRADCGITSASYHQGVLSATILYEILLGKATLYAVLVSGLVLMAMVKKKNS

SEQ ID NO: 13 - protein, 27 aa, Artificial Sequence
  Synthetic
RAKRSGSGATNFSLLKQAGDVEENPGP

SEQ ID NO: 14 - DNA, 81 bp, Artificial Sequence
  Synthetic
agggccaaacgctcagggagcggagctaccaatttttctctgctgaagcaggccggcgatgtggaggaaaatcctgggcca

SEQ ID NO: 15 - DNA, 825 bp, Artificial Sequence
  Synthetic
atgacactgaaaatggactcaagccctggattcgtggctgtcatcctgctgattctgggccggactcacggggatagcgtgacccagacagagggccaggtgaccgtctccgaatctaagagtctgatcattaactgtacctactccgccacatctatcgggtatcctaatctgttctggtacgtgcgctatccaggcgaggggctgcagctgctgctgaaagtcattaccgctgggcagaagggatcctctcgaggattcgaggcaacatacaacaaagaagccacttcatttcatctgcagaaggcaagcgtgcaggaatcagatagcgccgtgtactattgcgcactgtggtccggctcttggcagctgatctttggatccggcacccagctgacagtgatgcccgacattcagaaccccgagcctgccgtctatcagctgaaggaccctcgaagtcaggatagcaccctgtgcctgttcaccgactttgattcccagatcaatgtgcccaaaacaatggaatctggcactttcattaccgacaagacagtcctggatatgaaagctatggacagtaagtcaaacggggcaatcgcctggagcaatcagacttccttcacctgccaggatatcttcaaggagacaaacgcaacttaccccagttcagacgtgccttgtgatgccactctgaccgagaagagcttcgaaaccgacatgaacctgaattttcagaatctgagcgtgatgggcctgcgcatcctgctgctgaaggtggctgggttcaatctgctgatgacactgagactgtggagtagttgataa

SEQ ID NO: 16 - DNA, 909 bp, Artificial Sequence
  Synthetic
atggccacacgcctgctgtgctacactgtgctgtgcctgctgggggctcgcatcctgaactcaaaagtcatccagacacctcgctacctggtcaaaggccaggggcagaaagccaagatgagatgcatccctgagaaggggcacccagtggtcttctggtaccagcagaacaaaaacaatgagttcaagtttctgatcaactttcagaatcaggaagtgctgcagcagattgatatgaccgagaagcggttctcagccgaatgcccaagcaattccccctgtagcctggagatccagagctccgaagccggcgatagcgccctgtacctgtgcgctagcagagactccccagagcagtattttggacccggcacaagactgactgtgctggaagacctgaggaacgtgactccccctaaagtctctctgttcgagcctagtaaggctgaaatcgcaaacaagcagaaggccaccctggtgtgcctggctaggggcttctttccagatcacgtggagctgtcctggtgggtcaacgggaaagaagtgcattctggagtcagtacagacccccaggcttacaaggagtcaaattacagctattgcctgtctagtcggctgagagtgtctgcaactttttggcacaacccacgaaatcatttccggtgtcaggtgcagtttcacggactgtccgaggaagataaatggcccgagggctctccaaagcccgtgacacagaacatcagtgccgaagcttggggacgagctgactgcggaattacttctgcaagttatcatcagggcgtgctgtccgcaaccatcctgtacgagattctgctggggaaggcaacactgtatgccgtgctggtcagtggactggtgctgatggctatggtgaagaagaagaacagc

SEQ ID NO: 17 - DNA, 1815 bp, Artificial Sequence
  Synthetic
atggccctgaaaatggactctagccctgggtttgtcgccgtcatcctgctgatcctggggagaactcacggagatagcgtcactcagaccgaaggacaggtgacagtcagcgagtccaagtctctgatcattaactgcacatacagcgccacttccatcggctatcctaatctgttttggtacgtgaggtatccaggcgaagggctgcagctgctgctgaaggtcattactgctgggcagaaaggaagctcccgcggcttcgaggctacttacaacaaggaagcaacctcatttcacctgcagaaagcaagcgtgcaggagagtgattcagcagtctactattgcgcactgtggagcggatcctggcagctgatctttggaagcggcactcagctgaccgtgatgcccgacattcagaacccagagcccgccgtctatcagctgaaggaccctaggtctcaggatagcaccctgtgcctgttcacagactttgattcacagatcaatgtgcctaagacaatggagtccggcacattcattactgacaaaaccgtcctggatatgaaggctatggactctaaaagtaacggggccatcgcttggagcaatcagacatccttcacttgccaggatatcttcaaggagaccaacgccacatacccttctagtgacgtgccatgtgatgctaccctgacagagaaaagcttcgaaaccgacatgaacctgaattttcagaacctgtccgtgatgggcctgcggatcctgctgctgaaggtcgccgggtttaatctgctgatgactctgagactgtggtcaagcagggcaaagcggagcggaagcggagcaaccaacttctctctgctgaaacaggcaggggatgtggaggaaaatcctggaccaatggccacacggctgctgtgctacaccgtgctgtgcctgctgggagcacgcatcctgaatagcaaagtgatccagacaccccgatatctggtcaaaggccaggggcagaaggccaaaatgagatgcatccccgagaagggacatcctgtggtcttctggtatcagcagaacaagaacaacgagttcaaatttctgatcaacttccagaatcaggaagtgctgcagcagattgatatgaccgagaaacgattctctgccgaatgcccatccaattctccctgtagtctggagatccagtcctctgaagccggcgatagcgccctgtacctgtgcgcttcacgcgacagcccagagcagtattttggacccggcactagactgaccgtgctggaagacctgaggaacgtgaccccccctaaggtctctctgttcgagcctagtaaagctgaaattgcaaataagcagaaagccaccctggtgtgcctggctaggggcttctttccagatcacgtggagctgtcctggtgggtcaacggaaaggaagtgcattccggcgtctctactgacccccaggcctacaaagagagtaattactcatattgcctgagttcacggctgagagtgtctgctaccttctggcacaacccacgaaatcatttccggtgtcaggtgcagtttcacggactgtccgaggaggataagtggcccgagggctctcccaaacctgtgacacagaacatcagtgcagaagcatggggacgagctgactgtggaattactagtgcatcataccatcagggggtgctgtccgctaccatcctgtatgagattctgctgggaaaggcaacactgtatgctgtgctggtgtctgggctggtgctgatggctatggtgaaaaagaagaactcatgataa

SEQ ID NO: 18 - DNA, 1815 bp, Artificial Sequence
  Synthetic
atggccacacgcctgctgtgctacactgtgctgtgcctgctgggggctcgcatcctgaactcaaaagtcatccagacacctcgctacctggtcaaaggccaggggcagaaagccaagatgagatgcatccctgagaaggggcacccagtggtcttctggtaccagcagaacaaaaacaatgagttcaagtttctgatcaactttcagaatcaggaagtgctgcagcagattgatatgaccgagaagcggttctcagccgaatgcccaagcaattccccctgtagcctggagatccagagctccgaagccggcgatagcgccctgtacctgtgcgctagcagagactccccagagcagtattttggacccggcacaagactgactgtgctggaagacctgaggaacgtgactccccctaaagtctctctgttcgagcctagtaaggctgaaatcgcaaacaagcagaaggccaccctggtgtgcctggctaggggcttctttccagatcacgtggagctgtcctggtgggtcaacgggaaagaagtgcattctggagtcagtacagacccccaggcttacaaggagtcaaattacagctattgcctgtctagtcggctgagagtgtctgcaactttttggcacaacccacgaaatcatttccggtgtcaggtgcagtttcacggactgtccgaggaagataaatggcccgagggctctccaaagcccgtgacacagaacatcagtgccgaagcttggggacgagctgactgcggaattacttctgcaagttatcatcagggcgtgctgtccgcaaccatcctgtacgagattctgctggggaaggcaacactgtatgccgtgctggtcagtggactggtgctgatggctatggtgaagaagaagaacagcagggccaaacgctcagggagcggagctaccaatttttctctgctgaagcaggccggcgatgtggaggaaaatcctgggccaatgacactgaaaatggactcaagccctggattcgtggctgtcatcctgctgattctgggccggactcacggggatagcgtgacccagacagagggccaggtgaccgtctccgaatctaagagtctgatcattaactgtacctactccgccacatctatcgggtatcctaatctgttctggtacgtgcgctatccaggcgaggggctgcagctgctgctgaaagtcattaccgctgggcagaagggatcctctcgaggattcgaggcaacatacaacaaagaagccacttcatttcatctgcagaaggcaagcgtgcaggaatcagatagcgccgtgtactattgcgcactgtggtccggctcttggcagctgatctttggatccggcacccagctgacagtgatgcccgacattcagaaccccgagcctgccgtctatcagctgaaggaccctcgaagtcaggatagcaccctgtgcctgttcaccgactttgattcccagatcaatgtgcccaaaacaatggaatctggcactttcattaccgacaagacagtcctggatatgaaagctatggacagtaagtcaaacggggcaatcgcctggagcaatcagacttccttcacctgccaggatatcttcaaggagacaaacgcaacttaccccagttcagacgtgccttgtgatgccactctgaccgagaagagcttcgaaaccgacatgaacctgaattttcagaatctgagcgtgatgggcctgcgcatcctgctgctgaaggtggctgggttcaatctgctgatgacactgagactgtggagtagttgataa

SEQ ID NO: 19 - DNA, 822 bp, Mus musculus
atgacactaaagatggactcttctccaggcttcgtggctgtgatacttctcatactgggaaggacccatggagattccgtgactcaaacagaaggccaagtgactgtctcagaaagcaagtccctgataataaattgcacgtattcagccacaagcataggttaccctaatcttttctggtatgttcgatatcctggagaaggtctacaactcctcctgaaagtcattacggctggccagaagggaagcagcagagggtttgaagccacatacaataaagaagccacctccttccacttgcagaaagcctcagtgcaagagtcagactcggctgtgtactactgcgctctgtggtctggcagctggcaactcatctttggatctggaacccaactgacagttatgcctgacatccagaacccagaacctgctgtgtaccagttaaaagatcctcggtctcaggacagcaccctctgcctgttcaccgactttgactcccaaatcaatgtgccgaaaaccatggaatctggaacgttcatcactgacaaaactgtgctggacatgaaagctatggattccaagagcaatggggccattgcctggagcaaccagacaagcttcacctgccaagatatcttcaaagagaccaacgccacctaccccagttcagacgttccctgtgatgccacgttgactgagaaaagctttgaaacagatatgaacctaaactttcaaaacctgtcagttatgggactccgaatcctcctgctgaaagtagccggatttaacctgctcatgacgctgaggctgtggtccagttga

SEQ ID NO: 20 - DNA, 912 bp, Mus musculus
atggctacaaggctcctctgttacacagtactttgtctcctgggtgcaagaattttgaattcaaaagtcattcagactccaagatatctggtgaaagggcaaggacaaaaagcaaagatgaggtgtatccctgaaaagggacatccagttgtattctggtatcaacaaaataagaacaatgagtttaaatttttgattaactttcagaatcaagaagttcttcagcaaatagacatgactgaaaaacgattctctgctgagtgtccttcaaactcaccttgcagcctagaaattcagtcctctgaggcaggagactcagcactgtacctctgtgccagcagggacagtcctgaacagtacttcggtcccggcaccaggctcacggttttagaggatctgagaaatgtgactccacccaaggtctccttgtttgagccatcaaaagcagagattgcaaacaaacaaaaggctaccctcgtgtgcttggccaggggcttcttccctgaccacgtggagctgagctggtgggtgaatggcaaggaggtccacagtggggtcagcacggaccctcaggcctacaaggagagcaattatagctactgcctgagcagccgcctgagggtctctgctaccttctggcacaatcctcgaaaccacttccgctgccaagtgcagttccatgggctttcagaggaggacaagtggccagagggctcacccaaacctgtcacacagaacatcagtgcagaggcctggggccgagcagactgtggaatcacttcagcatcctatcatcagggggttctgtctgcaaccatcctctatgagatcctactggggaaggccaccctatatgctgtgctggtcagtggcctggtgctgatggccatggtcaagaaaaaaaattcctga

SEQ ID NO: 21 - DNA, 408 bp, Artificial Sequence
  Synthetic
atgacactgaaaatggactcaagccctggattcgtggctgtcatcctgctgattctgggccggactcacggggatagcgtgacccagacagagggccaggtgaccgtctccgaatctaagagtctgatcattaactgtacctactccgccacatctatcgggtatcctaatctgttctggtacgtgcgctatccaggcgaggggctgcagctgctgctgaaagtcattaccgctgggcagaagggatcctctcgaggattcgaggcaacatacaacaaagaagccacttcatttcatctgcagaaggcaagcgtgcaggaatcagatagcgccgtgtactattgcgcactgtggtccggctcttggcagctgatctttggatccggcacccagctgacagtgatgccc

SEQ ID NO: 22 - DNA, 393 bp, Artificial Sequence
  Synthetic
atggccacacgcctgctgtgctacactgtgctgtgcctgctgggggctcgcatcctgaactcaaaagtcatccagacacctcgctacctggtcaaaggccaggggcagaaagccaagatgagatgcatccctgagaaggggcacccagtggtcttctggtaccagcagaacaaaaacaatgagttcaagtttctgatcaactttcagaatcaggaagtgctgcagcagattgatatgaccgagaagcggttctcagccgaatgcccaagcaattccccctgtagcctggagatccagagctccgaagccggcgatagcgccctgtacctgtgcgctagcagagactccccagagcagtattttggacccggcacaagactgactgtgctggaa

SEQ ID NO: 23 - protein, 9 aa, Artificial Sequence
  Synthetic
SLAMWITQC

SEQ ID NO: 24 - protein, 9 aa, Artificial Sequence
  Synthetic
SLLAWITQC

SEQ ID NO: 25 - protein, 9 aa, Artificial Sequence
  Synthetic
SLLMAITQC

SEQ ID NO: 26 - protein, 9 aa, Artificial Sequence
  Synthetic
SLLMWATQC

SEQ ID NO: 27 - protein, 9 aa, Artificial Sequence
  Synthetic
SLLMWIAQC

SEQ ID NO: 28 - protein, 9 aa, Artificial Sequence
  Synthetic
SLLMWITAC